European Patent Specification EP 3 713 644 B1, published August 7, 2024. Title: COMPOSITIONS AND METHODS FOR MODULATING HIF-2A TO IMPROVE MUSCLE GENERATION AND REPAIR. Applicant: University of Georgia Research Foundation, Inc. YIN, HANG XIE, LIWEI. The sequence listing filed with the application follows.

SEQUENCE LISTING (39 sequences)

SEQ ID NO: 1 - DNA, 5184 bp, Homo sapiens
gctttacactcgcgagcggaccgccacacgggtccggtgcccgctgcgcttccgccccagcgctcctgaggcggccgtacaatcctcggcagtgtcctgagactgtatggtcagctcagcccggcctccgactccttccgactcccagcattcgagccacttttttttttctttgaaaactcagaaaagtgactccttttccagggaaaaaggaacttgggttcccttctctccgtcctcttttcgggtctgacagcctccacccactccttccccggaccccgcctccgcgcgcaggttcctcccagtcacctttctccacccccgcccccgcacctagcccgccgcgcgccaccttccacctgactgcgcggggcgctcgggacctgcgcgcacctcggaccttcaccacccgcccgggccgcggggagcggacgagggccacagccccccacccgccagggagcccaggtgctcggcgtctgaacgtctcaaagggccacagcgacaatgacagctgacaaggagaagaaaaggagtagctcggagaggaggaaggagaagtcccgggatgctgcgcggtgccggcggagcaaggagacggaggtgttctatgagctggcccatgagctgcctctgccccacagtgtgagctcccatctggacaaggcctccatcatgcgactggcaatcagcttcctgcgaacacacaagctcctctcctcagtttgctctgaaaacgagtccgaagccgaagctgaccagcagatggacaacttgtacctgaaagccttggagggtttcattgccgtggtgacccaagatggcgacatgatctttctgtcagaaaacatcagcaagttcatgggacttacacaggtggagctaacaggacatagtatctttgacttcactcatccctgcgaccatgaggagattcgtgagaacctgagtctcaaaaatggctctggttttgggaaaaaaagcaaagacatgtccacagagcgggacttcttcatgaggatgaagtgcacggtcaccaacagaggccgtactgtcaacctcaagtcagccacctggaaggtcttgcactgcacgggccaggtgaaagtctacaacaactgccctcctcacaatagtctgtgtggctacaaggagcccctgctgtcctgcctcatcatcatgtgtgaaccaatccagcacccatcccacatggacatccccctggatagcaagaccttcctgagccgccacagcatggacatgaagttcacctactgtgatgacagaatcacagaactgattggttaccaccctgaggagctgcttggccgctcagcctatgaattctaccatgcgctagactccgagaacatgaccaagagtcaccagaacttgtgcaccaagggtcaggtagtaagtggccagtaccggatgctcgcaaagcatgggggctacgtgtggctggagacccaggggacggtcatctacaaccctcgcaacctgcagccccagtgcatcatgtgtgtcaactacgtcctgagtgagattgagaagaatgacgtggtgttctccatggaccagactgaatccctgttcaagccccacctgatggccatgaacagcatctttgatagcagtggcaagggggctgtgtctgagaagagtaacttcctattcaccaagctaaaggaggagcccgaggagctggcccagctggctcccaccccaggagacgccatcatctctctggatttcgggaatcagaacttcgaggagtcctcagcctatggcaaggccatcctgcccccgagccagccatgggccacggagttgaggagccacagcacccagagcgaggctgggagcctgcctgccttcaccgtgccccaggcagctgccccgggcagcaccacccccagtgccaccagcagcagcagcagctgctccacgcccaatagccctgaagactattacacatctttggataacgacctgaagattgaagtgattgagaagctcttcgccatggacacagaggccaaggaccaatgcagtacccagacggatttcaatgagctggacttggagacactggcaccctatatccccatggacggggaagacttccagctaagccccatctgccccgaggagcggctcttggcggagaacccacagtccaccccccagcactgcttcagtgccatgacaaacatcttccagccactggcccctgtagccccgcacagtcccttcctcctggacaagtttcagcagcagctggagagcaagaagacagagcccgagcaccggcccatgtcctccatcttctttgatgccggaagcaaagcatccctgccaccgtgctgtggccaggccagcacccctctctcttccatggggggcagatccaatacccagtggcccccagatccaccattacattttgggcccacaaagtgggccgtcggggatcagcgcacagagttcttgggagcagcgccgttggggccccctgtctctccaccccatgtctccaccttcaagacaaggtctgcaaagggttttggggctcgaggcccagacgtgctgagtccggccatggtagccctctccaacaagctgaagctgaagcgacagctggagtatgaagagcaagccttccaggacctgagcgggggggacccacctggtggcagcacctcacatttgatgtggaaacggatgaagaacctcaggggtgggagctgccctttgatgccggacaagccactgagcgcaaatgtacccaatgataagttcacccaaaaccccatgaggggcctgggccatcccctgagacatctgccgctgccacagcctccatctgccatcagtcccggggagaacagcaagagcaggttccccccacagtgctacgccacccagtaccaggactacagcctgtcgtcagcccacaaggtgtcaggcatggcaagccggctgctcgggccctcatttgagtcctacctgctgcccgaactgaccagatatgactgtgaggtgaacgtgcccgtgctgggaagctccacgctcctgcaaggaggggacctcctcagagccctggaccaggccacctgagccaggccttctacctgggcagcacctctgccgacgccgtcccaccagcttcactctctccgtctgtttttgcaactaggtatttctaacgccagcacactatttacaagatggacttacctggcagacttgcccaggtcaccaagcagtggcctttttctgagatgctcactttattatccctatttttaaagtacacaattgttttacctgttctgaaatgttcttaaattttgtaggatttttttcctccccaccttcaatgacttctaatttatattatccataggtttctctccctccttctccttctcacacacaactgtccatactaacaagtttggtgcatgtctgttcttctgtagggagaagctttagcttcattttactaaaaagattcctcgttattgttgttgccaaagagaaacaaaaatgattttgctttccaagcttggtttgtggcgtctccctcgcagagcccttctcgtttcttttttaaactaatcaccatattgtaaatttcagggtttttttttttttgtttaagctgactctttgctctaattttggaaaaaaagaaatgtgaagggtcaactccaacgtatgtggttatctgtgaaagttgcacagcgtggcttttcctaaactggtgtttttcccccgcatttggtggattttttattattattcaaaaacataactgagttttttaaaagaggagaaaatttatatctgggttaagtgtttatcatatatatgggtactttgtaatatctaaaaacttagaaacggaaatggaatcctgctcacaaaatcactttaagatcttttcgaagctgttaatttttcttagtgttgtggacactgcagacttgtccagtgctcccacggcctgtacggacactgtggaaggcctccctctgtcggctttttgccatctgtgatatgccataggtgtgacaatccgagcagtggagtcattcagcgggagcactgcgcgctatcccctcacattctctatgtactatgtatgtatgtattattattattgctgccaagagggtctgatggcacgttgtggggtcggggggtggggcggggaagtgctctaacttttcttaaggttttgttgctagcccttcaagtgcactgagctatgtgactcggatggtctttcacacggcacatttggacatttccagaactaccatgagatggtttagacgggaattcatgcaaatgaggggtcaaaaatggtatagtgaccccgtccacgtcctccaagctcacgaccttggagccccgtggagctggactgaggaggaggctgcacagcgggagagcagctggtccagaccagccctgcagcccccactcagccggcagccagatggccccgcaaggcctccagggatggcccctagccacaggccctggctgaggtctctgggtcggtcagtgacatgtaggtaggaagcactgaaaatagtgttcccagagcactttgcaactccctgggtaagagggacgacacctctggtttttcaataccaattacatggaacttttctgtaatgggtacaatgaagaagtttctaaaaacacacacaaagcacattgggccaactatttagtaagcccggatagacttattgccaaaaacaaaaaatagctttcaaaagaaatttaagttctatgagaaattccttagtcatggtgttgcgtaaatcatattttagctgcacggcattaccccacacagggtggcagaacttgaagggttactgacgtgtaaatgctggtatttgatttcctgtgtgtgttgccctggcattaagggcattttacccttgcagttttactaaaacactgaaaaatattccaagcttcatattaaccctacctgtcaacgtaacgatttcatgaacgttattatattgtcgaattcctactgacaacattataactgtatgggagcttaactttataaggaaatgtattttgacactggtatcttattaaagtattctgatcctaccactgaaaaaaaaaaaaaaaaaa

SEQ ID NO: 2 - protein, 870 aa, Homo sapiens
MTADKEKKRSSSERRKEKSRDAARCRRSKETEVFYELAHELPLPHSVSSHLDKASIMRLAISFLRTHKLLSSVCSENESEAEADQQMDNLYLKALEGFIAVVTQDGDMIFLSENISKFMGLTQVELTGHSIFDFTHPCDHEEIRENLSLKNGSGFGKKSKDMSTERDFFMRMKCTVTNRGRTVNLKSATWKVLHCTGQVKVYNNCPPHNSLCGYKEPLLSCLIIMCEPIQHPSHMDIPLDSKTFLSRHSMDMKFTYCDDRITELIGYHPEELLGRSAYEFYHALDSENMTKSHQNLCTKGQVVSGQYRMLAKHGGYVWLETQGTVIYNPRNLQPQCIMCVNYVLSEIEKNDVVFSMDQTESLFKPHLMAMNSIFDSSGKGAVSEKSNFLFTKLKEEPEELAQLAPTPGDAIISLDFGNQNFEESSAYGKAILPPSQPWATELRSHSTQSEAGSLPAFTVPQAAAPGSTTPSATSSSSSCSTPNSPEDYYTSLDNDLKIEVIEKLFAMDTEAKDQCSTQTDFNELDLETLAPYIPMDGEDFQLSPICPEERLLAENPQSTPQHCFSAMTNIFQPLAPVAPHSPFLLDKFQQQLESKKTEPEHRPMSSIFFDAGSKASLPPCCGQASTPLSSMGGRSNTQWPPDPPLHFGPTKWAVGDQRTEFLGAAPLGPPVSPPHVSTFKTRSAKGFGARGPDVLSPAMVALSNKLKLKRQLEYEEQAFQDLSGGDPPGGSTSHLMWKRMKNLRGGSCPLMPDKPLSANVPNDKFTQNPMRGLGHPLRHLPLPQPPSAISPGENSKSRFPPQCYATQYQDYSLSSAHKVSGMASRLLGPSFESYLLPELTRYDCEVNVPVLGSSTLLQGGDLLRALDQAT

SEQ ID NO: 3 - protein, 11 aa, Artificial Sequence
  synthetic polypeptide
YGRKKRRQRRR

SEQ ID NO: 4 - protein, 9 aa, Artificial Sequence
  synthetic polypeptide
RKKRRQRRR

SEQ ID NO: 5 - protein, 7 aa, Artificial Sequence
  synthetic polypeptide
RRRRRRR

SEQ ID NO: 6 - protein, 12 aa, Artificial Sequence
  synthetic polypeptide
RRQRRTSKLMKR

SEQ ID NO: 7 - protein, 27 aa, Artificial Sequence
  synthetic polypeptide
GWTLNSAGYLLGKINLKALAALAKKIL

SEQ ID NO: 8 - protein, 29 aa, Artificial Sequence
  synthetic polypeptide
WEAKLAKALAKALAKHLAKALAKALKCEA

SEQ ID NO: 9 - protein, 16 aa, Artificial Sequence
  synthetic polypeptide
RQIKIWFQNRRMKWKK

SEQ ID NO: 10 - protein, 7 aa, Artificial Sequence
  synthetic polypeptide
PKKKRKV

SEQ ID NO: 11 - protein, 7 aa, Artificial Sequence
  synthetic polypeptide
GKKRSKV

SEQ ID NO: 12 - protein, 7 aa, Artificial Sequence
  synthetic polypeptide
KSRKRKL

SEQ ID NO: 13 - protein, 19 aa, Artificial Sequence
  synthetic polypeptide
KRPAATKKAGQAKKKKLDK

SEQ ID NO: 14 - protein, 20 aa, Artificial Sequence
  synthetic polypeptide
RKKRKTEEESPLKDKAKKSK

SEQ ID NO: 15 - protein, 20 aa, Artificial Sequence
  synthetic polypeptide
KDCVMNKHHRNRCQYCRLQR

SEQ ID NO: 16 - protein, 9 aa, Artificial Sequence
  syntehtic polypeptide
PAAKRVKLD

SEQ ID NO: 17 - protein, 20 aa, Artificial Sequence
  syntehtic polypeptide
KKYENVVIKRSPRKRGRPRK

SEQ ID NO: 18 - DNA, 97 bp, Artificial Sequence
  synthetic polynucleotide
tgctgttgacagtgagcgaacacttgatgtggaaacgtattagtgaagccacagatgtaatacgtttccacatcaagtgtgtgcctactgcctcgga

SEQ ID NO: 19 - DNA, 97 bp, Artificial Sequence
  synthetic polynucleotide
tgctgttgacagtgagcgatccaacaagctgaagctaaagtagtgaagccacagatgtactttagcttcagcttgttggactgcctactgcctcgga

SEQ ID NO: 20 - DNA, 20 bp, Artificial Sequence
  synthetic polynucleotide
gagtgtcctgggttccttgc

SEQ ID NO: 21 - DNA, 20 bp, Artificial Sequence
  synthetic polynucleotide
ggcataatgcatttgcaagc

SEQ ID NO: 22 - DNA, 20 bp, Artificial Sequence
  synthetic polynucleotide
cccgtcactcaaccatttca

SEQ ID NO: 23 - DNA, 20 bp, Artificial Sequence
  synthetic polynucleotide
cttatcaatgggggctctgg

SEQ ID NO: 24 - DNA, 20 bp, Artificial Sequence
  synthetic polynucleotide
agatatggctggctttgtgc

SEQ ID NO: 25 - DNA, 19 bp, Artificial Sequence
  synthetic polynucleotide
gaactcgctcaggttctgc

SEQ ID NO: 26 - DNA, 18 bp, Artificial Sequence
  synthetic polynucleotide
acatggcccccgatgaat

SEQ ID NO: 27 - DNA, 20 bp, Artificial Sequence
  synthetic polynucleotide
caggtaaggctcgaacgatg

SEQ ID NO: 28 - DNA, 20 bp, Artificial Sequence
  synthetic polynucleotide
ggatttggccgagagttgtt

SEQ ID NO: 29 - DNA, 20 bp, Artificial Sequence
  synthetic polynucleotide
cggctaggagaaggacacta

SEQ ID NO: 30 - DNA, 20 bp, Artificial Sequence
  synthetic polynucleotide
cggcgggatcctataagttg

SEQ ID NO: 31 - DNA, 19 bp, Artificial Sequence
  synthetic polynucleotide
gcgtggataatggttggca

SEQ ID NO: 32 - DNA, 20 bp, Artificial Sequence
  synthetic polynucleotide
tcctctgacatttgcaggtc

SEQ ID NO: 33 - DNA, 18 bp, Artificial Sequence
  synthetic polynucleotide
aaggcattggctggaaga

SEQ ID NO: 34 - DNA, 20 bp, Artificial Sequence
  synthetic polynucleotide
cgccatgtctctagtgatcc

SEQ ID NO: 35 - DNA, 20 bp, Artificial Sequence
  synthetic polynucleotide
ggtcgatgtctgctttcctc

SEQ ID NO: 36 - DNA, 21 bp, Artificial Sequence
  synthetic polynucleotide
acttcgtgcaagaaatgctga

SEQ ID NO: 37 - DNA, 23 bp, Artificial Sequence
  synthetic polynucleotide
tctggattgttcttcactcttgg

SEQ ID NO: 38 - DNA, 5011 bp, Homo sapiens
cttttccagggaaaaaggaacttgggttcccttctctccgtcctcttttcgggtctgacagcctccacccactccttccccggaccccgcctccgcgcgcaggttcctcccagtcacctttctccacccccgcccccgcacctagcccgccgcgcgccaccttccacctgactgcgcggggcgctcgggacctgcgcgcacctcggaccttcaccacccgcccgggccgcggggagcggacgagggccacagccccccacccgccagggagcccaggtgctcggcgtctgaacgtctcaaagggccacagcgacaatgacagctgacaaggagaagaaaaggagtagctcggagaggaggaaggagaagtcccgggatgctgcgcggtgccggcggagcaaggagacggaggtgttctatgagctggcccatgagctgcctctgccccacagtgtgagctcccatctggacaaggcctccatcatgcgactggcaatcagcttcctgcgaacacacaagctcctctcctcagtttgctctgaaaacgagtccgaagccgaagctgaccagcagatggacaacttgtacctgaaagccttggagggtttcattgccgtggtgacccaagatggcgacatgatctttctgtcagaaaacatcagcaagttcatgggacttacacaggtggagctaacaggacatagtatctttgacttcactcatccctgcgaccatgaggagattcgtgagaacctgagtctcaaaaatggctctggttttgggaaaaaaagcaaagacatgtccacagagcgggacttcttcatgaggatgaagtgcacggtcaccaacagaggccgtactgtcaacctcaagtcagccacctggaaggtcttgcactgcacgggccaggtgaaagtctacaacaactgccctcctcacaatagtctgtgtggctacaaggagcccctgctgtcctgcctcatcatcatgtgtgaaccaatccagcacccatcccacatggacatccccctggatagcaagaccttcctgagccgccacagcatggacatgaagttcacctactgtgatgacagaatcacagaactgattggttaccaccctgaggagctgcttggccgctcagcctatgaattctaccatgcgctagactccgagaacatgaccaagagtcaccagaacttgtgcaccaagggtcaggtagtaagtggccagtaccggatgctcgcaaagcatgggggctacgtgtggctggagacccaggggacggtcatctacaaccctcgcaacctgcagccccagtgcatcatgtgtgtcaactacgtcctgagtgagattgagaagaatgacgtggtgttctccatggaccagactgaatccctgttcaagccccacctgatggccatgaacagcatctttgatagcagtggcaagggggctgtgtctgagaagagtaacttcctattcaccaagctaaaggaggagcccgaggagctggcccagctggctcccaccccaggagacgccatcatctctctggatttcgggaatcagaacttcgaggagtcctcagcctatggcaaggccatcctgcccccgagccagccatgggccacggagttgaggagccacagcacccagagcgaggctgggagcctgcctgccttcaccgtgccccaggcagctgccccgggcagcaccacccccagtgccaccagcagcagcagcagctgctccacgcccaatagccctgaagactattacacatctttggataacgacctgaagattgaagtgattgagaagctcttcgccatggacacagaggccaaggaccaatgcagtacccagacggatttcaatgagctggacttggagacactggcaccctatatccccatggacggggaagacttccagctaagccccatctgccccgaggagcggctcttggcggagaacccacagtccaccccccagcactgcttcagtgccatgacaaacatcttccagccactggcccctgtagccccgcacagtcccttcctcctggacaagtttcagcagcagctggagagcaagaagacagagcccgagcaccggcccatgtcctccatcttctttgatgccggaagcaaagcatccctgccaccgtgctgtggccaggccagcacccctctctcttccatggggggcagatccaatacccagtggcccccagatccaccattacattttgggcccacaaagtgggccgtcggggatcagcgcacagagttcttgggagcagcgccgttggggccccctgtctctccaccccatgtctccaccttcaagacaaggtctgcaaagggttttggggctcgaggcccagacgtgctgagtccggccatggtagccctctccaacaagctgaagctgaagcgacagctggagtatgaagagcaagccttccaggacctgagcgggggggacccacctggtggcagcacctcacatttgatgtggaaacggatgaagaacctcaggggtgggagctgccctttgatgccggacaagccactgagcgcaaatgtacccaatgataagttcacccaaaaccccatgaggggcctgggccatcccctgagacatctgccgctgccacagcctccatctgccatcagtcccggggagaacagcaagagcaggttccccccacagtgctacgccacccagtaccaggactacagcctgtcgtcagcccacaaggtgtcaggcatggcaagccggctgctcgggccctcatttgagtcctacctgctgcccgaactgaccagatatgactgtgaggtgaacgtgcccgtgctgggaagctccacgctcctgcaaggaggggacctcctcagagccctggaccaggccacctgagccaggccttctacctgggcagcacctctgccgacgccgtcccaccagcttcactctctccgtctgtttttgcaactaggtatttctaacgccagcacactatttacaagatggacttacctggcagacttgcccaggtcaccaagcagtggcctttttctgagatgctcactttattatccctatttttaaagtacacaattgttttacctgttctgaaatgttcttaaattttgtaggatttttttcctccccaccttcaatgacttctaatttatattatccataggtttctctccctccttctccttctcacacacaactgtccatactaacaagtttggtgcatgtctgttcttctgtagggagaagctttagcttcattttactaaaaagattcctcgttattgttgttgccaaagagaaacaaaaatgattttgctttccaagcttggtttgtggcgtctccctcgcagagcccttctcgtttcttttttaaactaatcaccatattgtaaatttcagggtttttttttttgtttaagctgactctttgctctaattttggaaaaaaagaaatgtgaagggtcaactccaacgtatgtggttatctgtgaaagttgcacagcgtggcttttcctaaactggtgtttttcccccgcatttggtggattttttattattattcaaaaacataactgagttttttaaaagaggagaaaatttatatctgggttaagtgtttatcatatatatgggtactttgtaatatctaaaaacttagaaacggaaatggaatcctgctcacaaaatcactttaagatcttttcgaagctgttaatttttcttagtgttgtggacactgcagacttgtccagtgctcccacggcctgtacggacactgtggaaggcctccctctgtcggctttttgccatctgtgatatgccataggtgtgacaatccgagcagtggagtcattcagcgggagcactgcgcgctatcccctcacattctctatgtactatgtatgtatgtattattattattgctgccaagagggtctgatggcacgttgtggggtcggggggtggggcggggaagtgctctaacttttcttaaggttttgttgctagcccttcaagtgcactgagctatgtgactcggatggtctttcacacggcacatttggacatttccagaactaccatgagatggtttagacgggaattcatgcaaatgaggggtcaaaaatggtatagtgaccccgtccacgtcctccaagctcacgaccttggagccccgtggagctggactgaggaggaggctgcacagcgggagagcagctggtccagaccagccctgcagcccccactcagccggcagccagatggccccgcaaggcctccagggatggcccctagccacaggccctggctgaggtctctgggtcggtcagtgacatgtaggtaggaagcactgaaaatagtgttcccagagcactttgcaactccctgggtaagagggacgacacctctggtttttcaataccaattacatggaacttttctgtaatgggtacaatgaagaagtttctaaaaacacacacaaagcacattgggccaactatttagtaagcccggatagacttattgccaaaaacaaaaaatagctttcaaaagaaatttaagttctatgagaaattccttagtcatggtgttgcgtaaatcatattttagctgcacggcattaccccacacagggtggcagaacttgaagggttactgacgtgtaaatgctggtatttgatttcctgtgtgtgttgccctggcattaagggcattttacccttgcagttttactaaaacactgaaaaatattccaagcttcatattaaccctacctgtcaacgtaacgatttcatgaacgttattatattgtcgaattcctactgacaacattataactgtatgggagcttaactttataaggaaatgtattttgacactggtatcttattaaagtattctgatcctaaaaaaaaaaaaaaaaaaaaaaaaaaaaaaaaaaaaaaaaaaaaaaaaa

SEQ ID NO: 39 - protein, 883 aa, Homo sapiens
MLGLFVFKTGTQRRNRRLPYARSSSERRKEKSRDAARCRRSKETEVFYELAHELPLPHSVSSHLDKASIMRLAISFLRTHKLLSSVCSENESEAEADQQMDNLYLKALEGFIAVVTQDGDMIFLSENISKFMGLTQVELTGHSIFDFTHPCDHEEIRENLSLKNGSGFGKKSKDMSTERDFFMRMKCTVTNRGRTVNLKSATWKVLHCTGQVKVYNNCPPHNSLCGYKEPLLSCLIIMCEPIQHPSHMDIPLDSKTFLSRHSMDMKFTYCDDRITELIGYHPEELLGRSAYEFYHALDSENMTKSHQNLCTKGQVVSGQYRMLAKHGGYVWLETQGTVIYNPRNLQPQCIMCVNYVLSEIEKNDVVFSMDQTESLFKPHLMAMNSIFDSSGKGAVSEKSNFLFTKLKEEPEELAQLAPTPGDAIISLDFGNQNFEESSAYGKAILPPSQPWATELRSHSTQSEAGSLPAFTVPQAAAPGSTTPSATSSSSSCSTPNSPEDYYTSLDNDLKIEVIEKLFAMDTEAKDQCSTQTDFNELDLETLAPYIPMDGEDFQLSPICPEERLLAENPQSTPQHCFSAMTNIFQPLAPVAPHSPFLLDKFQQQLESKKTEPEHRPMSSIFFDAGSKASLPPCCGQASTPLSSMGGRSNTQWPPDPPLHFGPTKWAVGDQRTEFLGAAPLGPPVSPPHVSTFKTRSAKGFGARGPDVLSPAMVALSNKLKLKRQLEYEEQAFQDLSGGDPPGGSTSHLMWKRMKNLRGGSCPLMPDKPLSANVPNDKFTQNPMRGLGHPLRHLPLPQPPSAISPGENSKSRFPPQCYATQYQDYSLSSAHKVSGMASRLLGPSFESYLLPELTRYDCEVNVPVLGSSTLLQGGDLLRALDQAT